European Patent Specification EP 3 699 190 B9, published October 4, 2023. Title: MICE EXPRESSING HUMANIZED MAJOR HISTOCOMPATIBILITY COMPLEX. Applicant: Regeneron Pharmaceuticals, Inc. Application EP. The sequence listing filed with the application follows.

SEQUENCE LISTING (33 sequences)

SEQ ID NO: 1 - DNA, 19 bp, Artificial Sequence
  Synthetic
cagaacgccaggctgtaac

SEQ ID NO: 2 - DNA, 20 bp, Artificial Sequence
  Synthetic
ggagagcagggtcagtcaac

SEQ ID NO: 3 - DNA, 24 bp, Artificial Sequence
  Synthetic
caccgccactcacagctccttaca

SEQ ID NO: 4 - DNA, 22 bp, Artificial Sequence
  Synthetic
gtgggcaccatcttcatcattc

SEQ ID NO: 5 - DNA, 22 bp, Artificial Sequence
  Synthetic
cttcctttccagggtgtgactc

SEQ ID NO: 6 - DNA, 23 bp, Artificial Sequence
  Synthetic
aggcctgcgatcaggtggcacct

SEQ ID NO: 7 - DNA, 17 bp, Artificial Sequence
  Synthetic
tgcggccgatcttagcc

SEQ ID NO: 8 - DNA, 18 bp, Artificial Sequence
  Synthetic
ttgaccgattccttgcgg

SEQ ID NO: 9 - DNA, 21 bp, Artificial Sequence
  Synthetic
acgagcgggttcggcccattc

SEQ ID NO: 10 - DNA, 140 bp, Artificial Sequence
  Synthetic
tttgtaaacaaagtctacccagagacagatgacagacttcagctccaatgctgattggttcctcacttgggaccaaccctctcgagtaccgttcgtataatgtatgctatacgaagttatatgcatccgggtaggggagg

SEQ ID NO: 11 - DNA, 140 bp, Artificial Sequence
  Synthetic
cctcgacctgcagccctaggataacttcgtataatgtatgctatacgaacggtagagctccacaggcatttgggtgggcagggatggacggtgactgggacaatcgggatggaagagcatagaatgggagttagggaaga

SEQ ID NO: 12 - DNA, 110 bp, Artificial Sequence
  Synthetic
tgctgattggttcctcacttgggaccaaccctaagctttatctatgtcgggtgcggagaaagaggtaatgaaatggcacaaggagatcacacacccaaaccaaactcgcc

SEQ ID NO: 13 - DNA, 96 bp, Artificial Sequence
  Synthetic
cacatcagtgaggctagaataaattaaaatcgctaatatgaaaatggggatttgtacctctgagtgtgaaggctgggaagactgctttcaagggac

SEQ ID NO: 14 - DNA, 150 bp, Artificial Sequence
  Synthetic
tccatcacttcactgggtagcacagctgtaactgtccagcctgggtaccgagctcggatccactagtaacggccgccagtgtgctggaattcgcccttgatcgagctccctgggctgcaggtggtgggcgttgcgggtggggccggttaa

SEQ ID NO: 15 - DNA, 80 bp, Artificial Sequence
  Synthetic
atctccatcagaagggcaccggtataacttcgtataaggtatcctatacgaagttatatgcatggcctccgcgccgggtt

SEQ ID NO: 16 - DNA, 90 bp, Artificial Sequence
  Synthetic
ataacttcgtataaggtatcctatacgaagttatctcgagtggcttacaggtaggtgcgtgaagcttctacaagcacagttgccccctgg

SEQ ID NO: 17 - DNA, 90 bp, Artificial Sequence
  Synthetic
ctgtttcttccctaactcccattctatgctcttccatcccgaccgcggcccaatctctctccactacttcctgcctacatgtatgtaggt

SEQ ID NO: 18 - DNA, 80 bp, Artificial Sequence
  Synthetic
caaggtttcctcctatgatgcttgtgtgaaactcggggccggccagcatttaacagtacagggatgggagcacagctcac

SEQ ID NO: 19 - DNA, 80 bp, Artificial Sequence
  Synthetic
gaaagcagtcttcccagccttcacactcagaggtacaaatccccattttcatattagcgattttaatttattctagcctc

SEQ ID NO: 20 - DNA, 80 bp, Artificial Sequence
  Synthetic
tcttccctaactcccattctatgctcttccatcccgaccgcggcccaatctctctccactacttcctgcctacatgtatg

SEQ ID NO: 21 - DNA, 21 bp, Artificial Sequence
  Synthetic
ctggcggcttgaagaatttgg

SEQ ID NO: 22 - DNA, 24 bp, Artificial Sequence
  Synthetic
catgatttccaggttggctttgtc

SEQ ID NO: 23 - DNA, 26 bp, Artificial Sequence
  Synthetic
cgatttgccagctttgaggctcaagg

SEQ ID NO: 24 - DNA, 20 bp, Artificial Sequence
  Synthetic
aggcttgggtgctccacttg

SEQ ID NO: 25 - DNA, 21 bp, Artificial Sequence
  Synthetic
gaccctggtgatgctggaaac

SEQ ID NO: 26 - DNA, 27 bp, Artificial Sequence
  Synthetic
caggtgtaaacctctccactccgagga

SEQ ID NO: 27 - DNA, 200 bp, Artificial Sequence
  Synthetic
ggattccccatctccacagtttcacttctgcacctaacctgggtcaggtccttctgtccggacactgttgacgcgcagtcagctcttacccccattgggtggcgcgatcacccaagaaccaatcagtgtcgccgcggacgctggatataaagtccacgcagcccgcagaactcagaagtcgcgaatcgccgacaggtgcg

SEQ ID NO: 28 - DNA, 200 bp, Artificial Sequence
  Synthetic
gtaaggagagtgtgggtgcagagctggggtcagggaaagctggagctttctgcagaccctgagctgctcagggctgagagctggggtcatgaccctcaccttcatttcttgtacctgtccttcccagagcctcctccatccactgtctccaacatggcgaccgttgctgttctggttgtccttggagctgcaatagtcac

SEQ ID NO: 29 - DNA, 149 bp, Artificial Sequence
  Synthetic
agtgtcgccgcggacgctggatataaagtccacgcagcccgcagaactcagaagtcgcgaatcgccgacaggtgcgatggccgtcatggcgccccgaaccctcgtcctgctactctcgggggctctggccctgacccagacctgggcgg

SEQ ID NO: 30 - DNA, 159 bp, Artificial Sequence
  Synthetic
ggtggtgccttctggacaggagcagagatacacctgccatgtgcagcatgagggtttgcccaagcccctcaccctgagatggggtaaggagagtgtgggtgcagagctggggtcagggaaagctggagctttctgcagaccctgagctgctcagggctg

SEQ ID NO: 31 - DNA, 27 bp, Artificial Sequence
  Synthetic
agtccttcagcctccactcaggtcagg

SEQ ID NO: 32 - DNA, 25 bp, Artificial Sequence
  Synthetic
taccaccagtacgcctacgacggca

SEQ ID NO: 33 - DNA, 18 bp, Artificial Sequence
  Synthetic
atcctgtaccagagagtg